European Patent Application EP 4 116 420 A1, published January 11, 2023. Title: USE OF GP73 INHIBITOR IN PREPARATION OF MEDICINE FOR TREATING DIABETES. Applicant: BEIJING SUNGEN BIOMEDICAL TECHNOLOGY CO. LTD. The sequence listing filed with the application follows.

SEQUENCE LISTING (9 sequences)

SEQ ID NO: 1 - RNA, 21 nt, Artificial sequence
ccugguggccuguguuauutt

SEQ ID NO: 2 - RNA, 21 nt, Artificial sequence
gcgagaagcucauucgagatt

SEQ ID NO: 3 - RNA, 21 nt, Artificial sequence
gcagaaugaggaaaccaautt

SEQ ID NO: 4 - RNA, 21 nt, Artificial sequence
ccaacaggcauccauccaatt

SEQ ID NO: 5 - RNA, 21 nt, Artificial sequence
caggagaugaauacgacautt

SEQ ID NO: 6 - RNA, 21 nt, Artificial sequence
gcagggaaugacagaaauatt

SEQ ID NO: 7 - RNA, 21 nt, Artificial sequence
ugugaaauggacagcgaaatt

SEQ ID NO: 8 - RNA, 21 nt, Artificial sequence
gcucuuaccgucagcauaatt

SEQ ID NO: 9 - RNA, 21 nt, Artificial sequence
gcaccuauggucuguguuutt